European Patent Specification EP 3 825 412 B1, published August 30, 2023. Title: NUCLEIC ACID SYNTHESIS AND SEQUENCING USING TETHERED NUCLEOSIDE TRIPHOSPHATES. Applicant: The Regents of the University of California. Application 17816338.2. The sequence listing filed with the application follows.

SEQUENCE LISTING (24 sequences)

SEQ ID NO: 1 - protein, 384 aa, Tarsius syrichta
MGHHHHHHHHHHSSGHIDDDDKHMSQYACQRRTTLNNHNQIFTDAFDILAENDEFRENEGPSLTFMRAASVLKSLPFTIISMKDIEGIPNLGDRVKSIIEEIIEDGESSAVKAVLNDERYKSFKLFTSVFGVGLKTSEKWFRMGFRTLSNIRSDKSLTFTRMQRAGFLYYEDLVSRVTRAEAEAVGVLVKEAVWASLPDAFVTMTGGFRRGKKTGHDVDFLITSPGATEEEEQQLLHKVISLWEHKGLLLYYDLVESTFEKLKLPSRKVDALDHFQKCFLILKLHHQRVDSDQSSWQEGKTWKAIRVDLVVCPYERRAFALLGWTGSRQFERDLRRYATHERKMIIDNHALYDKTKRIFLEAESEEEIFAHLGLDYIEPWERNA

SEQ ID NO: 2 - protein, 807 aa, Artificial Sequence
  Synthetic sequence
MGHHHHHHHHHHSSGHIDDDDKHMMKIEEGKLVIWINGDKGYNGLAEVGKKFEKDTGIKVTVEHPDKLEEKFPQVAATGDGPDIIFWAHDRFGGYAQSGLLAEITPDKAFQDKLYPFTWDAVRYNGKLIAYPIAVEALSLIYNKDLLPNPPKTWEEIPALDKELKAKGKSALMFNLQEPYFTWPLIAADGGYAFKYENGKYDIKDVGVDNAGAKAGLTFLVDLIKNKHMNADTDYSIAEAAFNKGETAMTINGPWAWSNIDTSKVNYGVTVLPTFKGQPSKPFVGVLSAGINAASPNKELAKEFLENYLLTDEGLEAVNKDKPLGAVALKSYEEELVKDPRIAATMENAQKGEIMPNIPQMSAFWYAVRTAVINAASGRQTVDEALKDAQTNSSSNNNNNNNNNNLGIEGRISHMSMGGRDIVDGSEFSPSPVPGSQNVPAPAVKKISQYACQRRTTLNNYNQLFTDALDILAENDELRENEGSALAFMRASSVLKSLPFPITSMKDTEGIPSLGDKVKSIIEGIIEDGESSEAKAVLNDERYKSFKLFTSVFGVGLKTAEKWFRMGFRTLSKIQSDKSLRFTQMQKAGFLYYEDLVSCVNRPEAEAVSMLVKEAVVTFLPDALVTMTGGFRRGKMTGHDVDFLITSPEATEDEEQQLLHKVTDFWKQQGLLLYADILESTFEKFKQPSRKVDALDHFQKCFLILKLDHGRVHSEKSGQQEGKGWKAIRVDLVMSPYDRRAFALLGWTGSRQFERDLRRYATHERKMMLDNHALYDRTKRVFLEAESEEEIFAHLGLDYIEPWERNA

SEQ ID NO: 3 - DNA, 46 bp, Artificial Sequence
  Syntthetic sequence
  Misc_feature (1)..(1): 5' phosphorylation at the 5' end
  Misc_feature (1)..(1): n is a uracil
  Misc_feature (22)..(22): n is a deoxythymidine nucleotide base modified with fluorescein
ntgaagagcgagagtgagtgancattaaagacgtgggcctggattt

SEQ ID NO: 4 - DNA, 59 bp, Artificial Sequence
  Synthetic sequence
gtgccgtgagacctggctcctgacgatatggataagctttgaagagcgagagtgagtga

SEQ ID NO: 5 - DNA, 56 bp, Artificial Sequence
  Syntthetic sequence
aaaagaattcaaaaaaaaaaaaaaaaaaaaaaaaaaaaaaaaaaaaaaaaaaaaaa

SEQ ID NO: 6 - DNA, 21 bp, Artificial Sequence
  Syntthetic sequence
  Misc_feature (1)..(1): phosphorylated at the 5' end
cattaaagacgtgggcgtgga

SEQ ID NO: 7 - DNA, 26 bp, Artificial Sequence
  Syntthetic sequence
  Misc_feature (4)..(4): n is a internal amino group labeled with Cy3 NHS
tttntgtgaaatccttccctcgatcc

SEQ ID NO: 8 - DNA, 42 bp, Artificial Sequence
  Synthetic sequence
  Misc_feature (1)..(1): aminohexyl modification of a 5' phosphate at the 5' end
cgactcacctcacgtcctcatgtgaaatccttccctcgatcc

SEQ ID NO: 9 - DNA, 30 bp, Artificial Sequence
  Syntthetic sequence
ttttgaattccaacacaccacccacccaac

SEQ ID NO: 10 - DNA, 30 bp, Artificial Sequence
  Syntthetic sequence
ttttaagcttcgactcacctcacgtcctca

SEQ ID NO: 11 - DNA, 47 bp, Artificial Sequence
  Syntthetic sequence
  Misc_feature (1)..(1): 5' phosphorylation at the 5' end
gcagccaactcagcttctgcaggggctttgttagcagccggatcctc

SEQ ID NO: 12 - DNA, 49 bp, Artificial Sequence
  Syntthetic sequence
aaacaagcgctcatgagccagaaatctggagcccgatcttccccatcgg

SEQ ID NO: 13 - DNA, 60 bp, Artificial Sequence
  Syntthetic sequence
gtgccgtgagacctggctcctgacgaggataagcttctatagtgagtcgtattaatttcg

SEQ ID NO: 14 - DNA, 40 bp, Artificial Sequence
  Syntthetic sequence
  Misc_feature (1)..(1): aminohexyl modification of a 5' phosphate at the 5' end
caacacaccacccacccaaccgcagatgtccgctttctgg

SEQ ID NO: 15 - DNA, 11 bp, Artificial Sequence
  Synthetic sequence
  Misc_Feature (1)..(1): linked to a -C tripple bond CCH2NH2
  Misc_Feature (2)..(2): linked to a -C tripple bond CCH2NH2
  Misc_Feature (3)..(3): linked to a -C tripple bond CCH2NH2
  Misc_Feature (4)..(4): linked to a -C tripple bond CCH2NH2
  Misc_Feature (11)..(11): OH group at the 3' end
ctagttttttt

SEQ ID NO: 16 - DNA, 11 bp, Artificial Sequence
  Synthetic sequence
  Misc_feature (11)..(11): OH group at the 3' end
ctagttttttt

SEQ ID NO: 17 - DNA, 11 bp, Artificial Sequence
  Synthetic sequence
tttctagtttt

SEQ ID NO: 18 - DNA, 10 bp, Artificial Sequence
  Synthetic sequence
ctactgactg

SEQ ID NO: 19 - DNA, 10 bp, Artificial Sequence
  Synthetic sequence
  Misc_feature (1)..(1): linked to a -C tripple bond CCH2NH2
  Misc_feature (1)..(1)
  Misc_feature (2)..(2): linked to a -C tripple bond CCH2NH2
  Misc_feature (3)..(3): linked to a -C tripple bond CCH2NH2
  Misc_feature (4)..(4): linked to a -C tripple bond CCH2NH2
  Misc_feature (5)..(5): linked to a -C tripple bond CCH2NH2
  Misc_feature (6)..(6): linked to a -C tripple bond CCH2NH2
  Misc_feature (7)..(7): linked to a -C tripple bond CCH2NH2
  Misc_feature (8)..(8): linked to a -C tripple bond CCH2NH2
  Misc_feature (9)..(9): linked to a -C tripple bond CCH2NH2
  Misc_feature (10)..(10): OH group at the 3' end
  Misc_feature (10)..(10): linked to a -C tripple bond CCH2NH2
ctactgactg

SEQ ID NO: 20 - DNA, 17 bp, Artificial Sequence
  Synthetic sequence
  Misc_feature (1)..(1): linked to a -C tripple bond CCH2NH2
  Misc_feature (2)..(2): linked to a -C tripple bond CCH2NH2
  Misc_feature (3)..(3): linked to a -C tripple bond CCH2NH2
  Misc_feature (4)..(4): linked to a -C tripple bond CCH2NH2
  Misc_feature (5)..(5): linked to a -C tripple bond CCH2NH2
  Misc_feature (6)..(6): linked to a -C tripple bond CCH2NH2
  Misc_feature (7)..(7): linked to a -C tripple bond CCH2NH2
  Misc_feature (8)..(8): linked to a -C tripple bond CCH2NH2
  Misc_feature (9)..(9): linked to a -C tripple bond CCH2NH2
  Misc_feature (10)..(10): linked to a -C tripple bond CCH2NH2
  Misc_feature (17)..(17): OH group at the 3' end
ctactgactgttttttt

SEQ ID NO: 21 - DNA, 17 bp, Artificial Sequence
  Synthetic sequence
ctactgactgttttttt

SEQ ID NO: 22 - DNA, 17 bp, Artificial Sequence
  Synthetic sequence
tttctactgactgtttt

SEQ ID NO: 23 - DNA, 11 bp, Artificial Sequence
  Synthetic sequence
aaaaaaactag

SEQ ID NO: 24 - DNA, 17 bp, Artificial Sequence
  Synthetic sequence
aaaaaaacagtcagtag